European Patent Specification EP 3 638 207 B1, published December 18, 2024. Title: NANOSTRUCTURED LIPID CARRIERS AND STABLE EMULSIONS AND USES THEREOF. Applicant: Infectious Disease Research Institute. The sequence listing filed with the application follows.

SEQUENCE LISTING (143 sequences)

SEQ ID NO: 1 - protein, 877 aa, Artificial Sequence
  Fusion protein ID91
MTINYQFGDVDAHGAMIRAQAGSLEAEHQAIISDVLTASDFWGGAGSAACQGFITQLGRNFQVIYEQANAHGQKVQAAGNNMAQTDSAVGSSWADDIDWDAIAQCESGGNWAANTGNGLYGGLQISQATWDSNGGVGSPAAASPQQQIEVADNIMKTQGPGAWPKCSSCSQGDAPLGSLTHILTFLAAETGGCSGSRDDVVDFGALPPEINSARMYAGPGSASLVAAAKMWDSVASDLFSAASAFQSVVWGLTVGSWIGSSAGLMAAAASPYVAWMSVTAGQAQLTAAQVRVAAAAYETAYRLTVPPPVIAENRTELMTLTATNLLGQNTPAIEANQAAYSQMWGQDAEAMYGYAATAATATEALLPFEDAPLITNPGGLLEQAVAVEEAIDTAAANQLMNNVPQALQQLAQPAQGVVPSSKLGGLWTAVSPHLSPLSNVSSIANNHMSMMGTGVSMTNTLHSMLKGLAPAAAQAVETAAENGVWAMSSLGSQLGSSLGSSGLGAGVAANLGRAASVGSLSVPPAWAAANQAVTPAARALPLTSLTSAAQTAPGHMLGGLPLGHSVNAGSGINNALRVPARAYAIPRTPAAGFSRPGLPVEYLQVPSPSMGRDIKVQFQSGGNNSPAVYLLDGLRAQDDYNGWDINTPAFEWYYQSGLSIVMPVGGQSSFYSDWYSPACGKAGCQTYKWETFLTSELPQWLSANRAVKPTGSAAIGLSMAGSSAMILAAYHPQQFIYAGSLSALLDPSQGMGPSLIGLAMGDAGGYKAADMWGPSSDPAWERNDPTQQIPKLVANNTRLWVYCGNGTPNELGGANIPAEFLENFVRSSNLKFQDAYNAAGGHNAVFNFPPNGTHSWEYWGAQLNAMKGDLQSSLGAG

SEQ ID NO: 2 - protein, 94 aa, Mycobacterium tuberculosis
MTINYQFGDVDAHGAMIRAQAGSLEAEHQAIISDVLTASDFWGGAGSAACQGFITQLGRNFQVIYEQANAHGQKVQAAGNNMAQTDSAVGSSWA

SEQ ID NO: 3 - protein, 105 aa, Mycobacterium tuberculosis
DDIDWDAIAQCESGGNWAANTGNGLYGGLQISQATWDSNGGVGSPAAASPQQQIEVADNIMKTQGPGAWPKCSSCSQGDAPLGSLTHILTFLAAETGGCSGSRDD

SEQ ID NO: 4 - protein, 393 aa, Mycobacterium tuberculosis
VVDFGALPPEINSARMYAGPGSASLVAAAKMWDSVASDLFSAASAFQSVVWGLTVGSWIGSSAGLMAAAASPYVAWMSVTAGQAQLTAAQVRVAAAAYETAYRLTVPPPVIAENRTELMTLTATNLLGQNTPAIEANQAAYSQMWGQDAEAMYGYAATAATATEALLPFEDAPLITNPGGLLEQAVAVEEAIDTAAANQLMNNVPQALQQLAQPAQGVVPSSKLGGLWTAVSPHLSPLSNVSSIANNHMSMMGTGVSMTNTLHSMLKGLAPAAAQAVETAAENGVWAMSSLGSQLGSSLGSSGLGAGVAANLGRAASVGSLSVPPAWAAANQAVTPAARALPLTSLTSAAQTAPGHMLGGLPLGHSVNAGSGINNALRVPARAYAIPRTPAAG

SEQ ID NO: 5 - protein, 285 aa, Mycobacterium tuberculosis
FSRPGLPVEYLQVPSPSMGRDIKVQFQSGGNNSPAVYLLDGLRAQDDYNGWDINTPAFEWYYQSGLSIVMPVGGQSSFYSDWYSPACGKAGCQTYKWETFLTSELPQWLSANRAVKPTGSAAIGLSMAGSSAMILAAYHPQQFIYAGSLSALLDPSQGMGPSLIGLAMGDAGGYKAADMWGPSSDPAWERNDPTQQIPKLVANNTRLWVYCGNGTPNELGGANIPAEFLENFVRSSNLKFQDAYNAAGGHNAVFNFPPNGTHSWEYWGAQLNAMKGDLQSSLGAG

SEQ ID NO: 6 - protein, 880 aa, Artificial Sequence
  pET29 vector
HMTINYQFGDVDAHGAMIRAQAGSLEAEHQAIISDVLTASDFWGGAGSAACQGFITQLGRNFQVIYEQANAHGQKVQAAGNNMAQTDSAVGSSWADDIDWDAIAQCESGGNWAANTGNGLYGGLQISQATWDSNGGVGSPAAASPQQQIEVADNIMKTQGPGAWPKCSSCSQGDAPLGSLTHILTFLAAETGGCSGSRDDVVDFGALPPEINSARMYAGPGSASLVAAAKMWDSVASDLFSAASAFQSVVWGLTVGSWIGSSAGLMAAAASPYVAWMSVTAGQAQLTAAQVRVAAAAYETAYRLTVPPPVIAENRTELMTLTATNLLGQNTPAIEANQAAYSQMWGQDAEAMYGYAATAATATEALLPFEDAPLITNPGGLLEQAVAVEEAIDTAAANQLMNNVPQALQQLAQPAQGVVPSSKLGGLWTAVSPHLSPLSNVSSIANNHMSMMGTGVSMTNTLHSMLKGLAPAAAQAVETAAENGVWAMSSLGSQLGSSLGSSGLGAGVAANLGRAASVGSLSVPPAWAAANQAVTPAARALPLTSLTSAAQTAPGHMLGGLPLGHSVNAGSGINNALRVPARAYAIPRTPAAGFSRPGLPVEYLQVPSPSMGRDIKVQFQSGGNNSPAVYLLDGLRAQDDYNGWDINTPAFEWYYQSGLSIVMPVGGQSSFYSDWYSPACGKAGCQTYKWETFLTSELPQWLSANRAVKPTGSAAIGLSMAGSSAMILAAYHPQQFIYAGSLSALLDPSQGMGPSLIGLAMGDAGGYKAADMWGPSSDPAWERNDPTQQIPKLVANNTRLWVYCGNGTPNELGGANIPAEFLENFVRSSNLKFQDAYNAAGGHNAVFNFPPNGTHSWEYWGAQLNAMKGDLQSSLGAGKL

SEQ ID NO: 7 - DNA, 2637 bp, Artificial Sequence
  Fusion protein ID91
accatcaactatcaattcggggacgtcgacgctcacggcgccatgatccgcgctcaggccgggtcgctggaggccgagcatcaggccatcatttctgatgtgttgaccgcgagtgacttttggggcggcgccggttcggcggcctgccaggggttcattacccagctgggccgtaacttccaggtgatctacgagcaggccaacgcccacgggcagaaggtgcaggctgccggcaacaacatggcacaaaccgacagcgccgtcggctccagctgggccgacgacatcgattgggacgccatcgcgcaatgcgaatccggcggcaattgggcggccaacaccggtaacgggttatacggtggtctgcagatcagccaggcgacgtgggattccaacggtggtgtcgggtcgccggcggccgcgagtccccagcaacagatcgaggtcgcagacaacattatgaaaacccaaggcccgggtgcgtggccgaaatgtagttcttgtagtcagggagacgcaccgctgggctcgctcacccacatcctgacgttcctcgcggccgagactggaggttgttcggggagcagggacgatgtggtggatttcggggcgttaccaccggagatcaactccgcgaggatgtacgccggcccgggttcggcctcgctggtggccgccgcgaagatgtgggacagcgtggcgagtgacctgttttcggccgcgtcggcgtttcagtcggtggtctggggtctgacggtggggtcgtggataggttcgtcggcgggtctgatggcggcggcggcctcgccgtatgtggcgtggatgagcgtcaccgcggggcaggcccagctgaccgccgcccaggtccgggttgctgcggcggcctacgagacagcgtataggctgacggtgcccccgccggtgatcgccgagaaccgtaccgaactgatgacgctgaccgcgaccaacctcttggggcaaaacacgccggcgatcgaggccaatcaggccgcatacagccagatgtggggccaagacgcggaggcgatgtatggctacgccgccacggcggcgacggcgaccgaggcgttgctgccgttcgaggacgccccactgatcaccaaccccggcgggctccttgagcaggccgtcgcggtcgaggaggccatcgacaccgccgcggcgaaccagttgatgaacaatgtgccccaagcgctgcaacagctggcccagccagcgcagggcgtcgtaccttcttccaagctgggtgggctgtggacggcggtctcgccgcatctgtcgccgctcagcaacgtcagttcgatagccaacaaccacatgtcgatgatgggcacgggtgtgtcgatgaccaacaccttgcactcgatgttgaagggcttagctccggcggcggctcaggccgtggaaaccgcggcggaaaacggggtctgggcgatgagctcgctgggcagccagctgggttcgtcgctgggttcttcgggtctgggcgctggggtggccgccaacttgggtcgggcggcctcggtcggttcgttgtcggtgccgccagcatgggccgcggccaaccaggcggtcaccccggcggcgcgggcgctgccgctgaccagcctgaccagcgccgcccaaaccgcccccggacacatgctgggcgggctaccgctggggcactcggtcaacgccggcagcggtatcaacaatgcgctgcgggtgccggcacgggcctacgcgataccccgcacaccggccgccggattctcccggccggggctgccggtcgagtacctgcaggtgccgtcgccgtcgatgggccgcgacatcaaggttcagttccagagcggtgggaacaactcacctgcggtttatctgctcgacggcctgcgcgcccaagacgactacaacggctgggatatcaacaccccggcgttcgagtggtactaccagtcgggactgtcgatagtcatgccggtcggcgggcagtccagcttctacagcgactggtacagcccggcctgcggtaaggctggctgccagacttacaagtgggaaaccttcctgaccagcgagctgccgcaatggttgtccgccaacagggccgtgaagcccaccggcagcgctgcaatcggcttgtcgatggccggctcgtcggcaatgatcttggccgcctaccacccccagcagttcatctacgccggctcgctgtcggccctgctggacccctctcaggggatggggcctagcctgatcggcctcgcgatgggtgacgccggcggttacaaggccgcagacatgtggggtccctcgagtgacccggcatgggagcgcaacgaccctacgcagcagatccccaagctggtcgcaaacaacacccggctatgggtttattgcgggaacggcaccccgaacgagttgggcggtgccaacatacccgccgagttcttggagaacttcgttcgtagcagcaacctgaagttccaggatgcgtacaacgccgcgggcgggcacaacgccgtgttcaacttcccgcccaacggcacgcacagctgggagtactggggcgctcagctcaacgccatgaagggtgacctgcagagttcgttaggcgccggctgaaagctt

SEQ ID NO: 8 - DNA, 279 bp, Mycobacterium tuberculosis
accatcaactatcaattcggggacgtcgacgctcacggcgccatgatccgcgctcaggccgggtcgctggaggccgagcatcaggccatcatttctgatgtgttgaccgcgagtgacttttggggcggcgccggttcggcggcctgccaggggttcattacccagctgggccgtaacttccaggtgatctacgagcaggccaacgcccacgggcagaaggtgcaggctgccggcaacaacatggcacaaaccgacagcgccgtcggctccagctgggcc

SEQ ID NO: 9 - DNA, 315 bp, Mycobacterium tuberculosis
gacgacatcgattgggacgccatcgcgcaatgcgaatccggcggcaattgggcggccaacaccggtaacgggttatacggtggtctgcagatcagccaggcgacgtgggattccaacggtggtgtcgggtcgccggcggccgcgagtccccagcaacagatcgaggtcgcagacaacattatgaaaacccaaggcccgggtgcgtggccgaaatgtagttcttgtagtcagggagacgcaccgctgggctcgctcacccacatcctgacgttcctcgcggccgagactggaggttgttcggggagcagggacgat

SEQ ID NO: 10 - DNA, 1179 bp, Mycobacterium tuberculosis
gtggtggatttcggggcgttaccaccggagatcaactccgcgaggatgtacgccggcccgggttcggcctcgctggtggccgccgcgaagatgtgggacagcgtggcgagtgacctgttttcggccgcgtcggcgtttcagtcggtggtctggggtctgacggtggggtcgtggataggttcgtcggcgggtctgatggcggcggcggcctcgccgtatgtggcgtggatgagcgtcaccgcggggcaggcccagctgaccgccgcccaggtccgggttgctgcggcggcctacgagacagcgtataggctgacggtgcccccgccggtgatcgccgagaaccgtaccgaactgatgacgctgaccgcgaccaacctcttggggcaaaacacgccggcgatcgaggccaatcaggccgcatacagccagatgtggggccaagacgcggaggcgatgtatggctacgccgccacggcggcgacggcgaccgaggcgttgctgccgttcgaggacgccccactgatcaccaaccccggcgggctccttgagcaggccgtcgcggtcgaggaggccatcgacaccgccgcggcgaaccagttgatgaacaatgtgccccaagcgctgcaacagctggcccagccagcgcagggcgtcgtaccttcttccaagctgggtgggctgtggacggcggtctcgccgcatctgtcgccgctcagcaacgtcagttcgatagccaacaaccacatgtcgatgatgggcacgggtgtgtcgatgaccaacaccttgcactcgatgttgaagggcttagctccggcggcggctcaggccgtggaaaccgcggcggaaaacggggtctgggcgatgagctcgctgggcagccagctgggttcgtcgctgggttcttcgggtctgggcgctggggtggccgccaacttgggtcgggcggcctcggtcggttcgttgtcggtgccgccagcatgggccgcggccaaccaggcggtcaccccggcggcgcgggcgctgccgctgaccagcctgaccagcgccgcccaaaccgcccccggacacatgctgggcgggctaccgctggggcactcggtcaacgccggcagcggtatcaacaatgcgctgcgggtgccggcacgggcctacgcgataccccgcacaccggccgccgga

SEQ ID NO: 11 - DNA, 855 bp, Mycobacterium tuberculosis
ttctcccggccggggctgccggtcgagtacctgcaggtgccgtcgccgtcgatgggccgcgacatcaaggttcagttccagagcggtgggaacaactcacctgcggtttatctgctcgacggcctgcgcgcccaagacgactacaacggctgggatatcaacaccccggcgttcgagtggtactaccagtcgggactgtcgatagtcatgccggtcggcgggcagtccagcttctacagcgactggtacagcccggcctgcggtaaggctggctgccagacttacaagtgggaaaccttcctgaccagcgagctgccgcaatggttgtccgccaacagggccgtgaagcccaccggcagcgctgcaatcggcttgtcgatggccggctcgtcggcaatgatcttggccgcctaccacccccagcagttcatctacgccggctcgctgtcggccctgctggacccctctcaggggatggggcctagcctgatcggcctcgcgatgggtgacgccggcggttacaaggccgcagacatgtggggtccctcgagtgacccggcatgggagcgcaacgaccctacgcagcagatccccaagctggtcgcaaacaacacccggctatgggtttattgcgggaacggcaccccgaacgagttgggcggtgccaacatacccgccgagttcttggagaacttcgttcgtagcagcaacctgaagttccaggatgcgtacaacgccgcgggcgggcacaacgccgtgttcaacttcccgcccaacggcacgcacagctgggagtactggggcgctcagctcaacgccatgaagggtgacctgcagagttcgttaggcgccggc

SEQ ID NO: 12 - DNA, 2643 bp, Artificial Sequence
  pET29 vector
catatgaccatcaactatcaattcggggacgtcgacgctcacggcgccatgatccgcgctcaggccgggtcgctggaggccgagcatcaggccatcatttctgatgtgttgaccgcgagtgacttttggggcggcgccggttcggcggcctgccaggggttcattacccagctgggccgtaacttccaggtgatctacgagcaggccaacgcccacgggcagaaggtgcaggctgccggcaacaacatggcacaaaccgacagcgccgtcggctccagctgggccgacgacatcgattgggacgccatcgcgcaatgcgaatccggcggcaattgggcggccaacaccggtaacgggttatacggtggtctgcagatcagccaggcgacgtgggattccaacggtggtgtcgggtcgccggcggccgcgagtccccagcaacagatcgaggtcgcagacaacattatgaaaacccaaggcccgggtgcgtggccgaaatgtagttcttgtagtcagggagacgcaccgctgggctcgctcacccacatcctgacgttcctcgcggccgagactggaggttgttcggggagcagggacgatgtggtggatttcggggcgttaccaccggagatcaactccgcgaggatgtacgccggcccgggttcggcctcgctggtggccgccgcgaagatgtgggacagcgtggcgagtgacctgttttcggccgcgtcggcgtttcagtcggtggtctggggtctgacggtggggtcgtggataggttcgtcggcgggtctgatggcggcggcggcctcgccgtatgtggcgtggatgagcgtcaccgcggggcaggcccagctgaccgccgcccaggtccgggttgctgcggcggcctacgagacagcgtataggctgacggtgcccccgccggtgatcgccgagaaccgtaccgaactgatgacgctgaccgcgaccaacctcttggggcaaaacacgccggcgatcgaggccaatcaggccgcatacagccagatgtggggccaagacgcggaggcgatgtatggctacgccgccacggcggcgacggcgaccgaggcgttgctgccgttcgaggacgccccactgatcaccaaccccggcgggctccttgagcaggccgtcgcggtcgaggaggccatcgacaccgccgcggcgaaccagttgatgaacaatgtgccccaagcgctgcaacagctggcccagccagcgcagggcgtcgtaccttcttccaagctgggtgggctgtggacggcggtctcgccgcatctgtcgccgctcagcaacgtcagttcgatagccaacaaccacatgtcgatgatgggcacgggtgtgtcgatgaccaacaccttgcactcgatgttgaagggcttagctccggcggcggctcaggccgtggaaaccgcggcggaaaacggggtctgggcgatgagctcgctgggcagccagctgggttcgtcgctgggttcttcgggtctgggcgctggggtggccgccaacttgggtcgggcggcctcggtcggttcgttgtcggtgccgccagcatgggccgcggccaaccaggcggtcaccccggcggcgcgggcgctgccgctgaccagcctgaccagcgccgcccaaaccgcccccggacacatgctgggcgggctaccgctggggcactcggtcaacgccggcagcggtatcaacaatgcgctgcgggtgccggcacgggcctacgcgataccccgcacaccggccgccggattctcccggccggggctgccggtcgagtacctgcaggtgccgtcgccgtcgatgggccgcgacatcaaggttcagttccagagcggtgggaacaactcacctgcggtttatctgctcgacggcctgcgcgcccaagacgactacaacggctgggatatcaacaccccggcgttcgagtggtactaccagtcgggactgtcgatagtcatgccggtcggcgggcagtccagcttctacagcgactggtacagcccggcctgcggtaaggctggctgccagacttacaagtgggaaaccttcctgaccagcgagctgccgcaatggttgtccgccaacagggccgtgaagcccaccggcagcgctgcaatcggcttgtcgatggccggctcgtcggcaatgatcttggccgcctaccacccccagcagttcatctacgccggctcgctgtcggccctgctggacccctctcaggggatggggcctagcctgatcggcctcgcgatgggtgacgccggcggttacaaggccgcagacatgtggggtccctcgagtgacccggcatgggagcgcaacgaccctacgcagcagatccccaagctggtcgcaaacaacacccggctatgggtttattgcgggaacggcaccccgaacgagttgggcggtgccaacatacccgccgagttcttggagaacttcgttcgtagcagcaacctgaagttccaggatgcgtacaacgccgcgggcgggcacaacgccgtgttcaacttcccgcccaacggcacgcacagctgggagtactggggcgctcagctcaacgccatgaagggtgacctgcagagttcgttaggcgccggctgaaagctt

SEQ ID NO: 13 - DNA, 60 bp, Artificial Sequence
  JEVss-FWD
gctggcctccctggctgtggtcattgcctgcgctggagcagccgaggtgaccaggagagg

SEQ ID NO: 14 - DNA, 59 bp, Artificial Sequence
  JEVss-REV
cacatgattgatccggcactcctcttgcccatggcggcggcgtgagctggcggcgggtg

SEQ ID NO: 15 - DNA, 56 bp, Artificial Sequence
  ZIKVss-FWD
ggaatcgtgggcctgctgctgaccacagcaatggcagccgaggtgaccaggagagg

SEQ ID NO: 16 - DNA, 54 bp, Artificial Sequence
  ZIKVss-REV
cacggatgtgtctgctcctctccgcatggcggcggcgtgagctggcggcgggtg

SEQ ID NO: 17 - DNA, 31 bp, Artificial Sequence
  ZIKV-prM-E-FWD
aatggactacgacatagtcgccgccgccatg

SEQ ID NO: 18 - DNA, 35 bp, Artificial Sequence
  ZIKV-prM-E-REV
gcggtttttgacaccgcggtcaggcagacacggcg

SEQ ID NO: 19 - protein, 15 aa, Artificial Sequence
  Id91 epitope 1
HMTINYQFGDVDAHG

SEQ ID NO: 20 - protein, 15 aa, Artificial Sequence
  Id91 epitope 2
FGDVDAHGAMIRAQA

SEQ ID NO: 21 - protein, 15 aa, Artificial Sequence
  Id91 epitope 3
GAMIRAQAGSLEAEH

SEQ ID NO: 22 - protein, 15 aa, Artificial Sequence
  Id91 epitope 4
AGSLEAEHQAIISDV

SEQ ID NO: 23 - protein, 15 aa, Artificial Sequence
  Id91 epitope 5
HQAIISDVLTASDFW

SEQ ID NO: 24 - protein, 15 aa, Artificial Sequence
  Id91 epitope 6
VLTASDFWGGAGSAA

SEQ ID NO: 25 - protein, 15 aa, Artificial Sequence
  Id91 epitope 7
WGGAGSAACQGFITQ

SEQ ID NO: 26 - protein, 15 aa, Artificial Sequence
  Id91 epitope 8
ACQGFITQLGRNFQV

SEQ ID NO: 27 - protein, 15 aa, Artificial Sequence
  Id91 epitope 9
QLGRNFQVIYEQANA

SEQ ID NO: 28 - protein, 15 aa, Artificial Sequence
  Id91 epitope 10
VIYEQANAHGQKVQA

SEQ ID NO: 29 - protein, 15 aa, Artificial Sequence
  Id91 epitope 11
AHGQKVQAAGNNMAQ

SEQ ID NO: 30 - protein, 15 aa, Artificial Sequence
  Id91 epitope 12
AAGNNMAQTDSAVGS

SEQ ID NO: 31 - protein, 15 aa, Artificial Sequence
  Id91 epitope 13
QTDSAVGSSWADDID

SEQ ID NO: 32 - protein, 15 aa, Artificial Sequence
  Id91 epitope 14
SSWADDIDWDAIAQC

SEQ ID NO: 33 - protein, 15 aa, Artificial Sequence
  Id91 epitope 15
DWDAIAQCESGGNWA

SEQ ID NO: 34 - protein, 15 aa, Artificial Sequence
  Id91 epitope 16
CESGGNWAANTGNGL

SEQ ID NO: 35 - protein, 15 aa, Artificial Sequence
  Id91 epitope 17
AANTGNGLYGGLQIS

SEQ ID NO: 36 - protein, 15 aa, Artificial Sequence
  Id91 epitope 18
LYGGLQISQATWDSN

SEQ ID NO: 37 - protein, 15 aa, Artificial Sequence
  Id91 epitope 19
SQATWDSNGGVGSPA

SEQ ID NO: 38 - protein, 15 aa, Artificial Sequence
  Id91 epitope 20
NGGVGSPAAASPQQQ

SEQ ID NO: 39 - protein, 15 aa, Artificial Sequence
  Id91 epitope 21
AAASPQQQIEVADNI

SEQ ID NO: 40 - protein, 15 aa, Artificial Sequence
  Id91 epitope 22
QIEVADNIMKTQGPG

SEQ ID NO: 41 - protein, 15 aa, Artificial Sequence
  Id91 epitope 23
IMKTQGPGAWPKCSS

SEQ ID NO: 42 - protein, 15 aa, Artificial Sequence
  Id91 epitope 24
GAWPKCSSCSQGDAP

SEQ ID NO: 43 - protein, 15 aa, Artificial Sequence
  Id91 epitope 25
SCSQGDAPLGSLTHI

SEQ ID NO: 44 - protein, 15 aa, Artificial Sequence
  Id91 epitope 26
PLGSLTHILTFLAAE

SEQ ID NO: 45 - protein, 15 aa, Artificial Sequence
  Id91 epitope 27
ILTFLAAETGGCSGS

SEQ ID NO: 46 - protein, 15 aa, Artificial Sequence
  Id91 epitope 28
ETGGCSGSRDDVVDF

SEQ ID NO: 47 - protein, 15 aa, Artificial Sequence
  Id91 epitope 29
SRDDVVDFGALPPEI

SEQ ID NO: 48 - protein, 15 aa, Artificial Sequence
  Id91 epitope 30
FGALPPEINSARMYA

SEQ ID NO: 49 - protein, 15 aa, Artificial Sequence
  Id91 epitope 31
INSARMYAGPGSASL

SEQ ID NO: 50 - protein, 15 aa, Artificial Sequence
  Id91 epitope 32
AGPGSASLVAAAKMW

SEQ ID NO: 51 - protein, 15 aa, Artificial Sequence
  Id91 epitope 33
LVAAAKMWDSVASDL

SEQ ID NO: 52 - protein, 15 aa, Artificial Sequence
  Id91 epitope 34
WDSVASDLFSAASAF

SEQ ID NO: 53 - protein, 15 aa, Artificial Sequence
  Id91 epitope 35
LFSAASAFQSVVWGL

SEQ ID NO: 54 - protein, 15 aa, Artificial Sequence
  Id91 epitope 36
FQSVVWGLTVGSWIG

SEQ ID NO: 55 - protein, 15 aa, Artificial Sequence
  Id91 epitope 37
LTVGSWIGSSAGLMA

SEQ ID NO: 56 - protein, 15 aa, Artificial Sequence
  Id91 epitope 38
GSSAGLMAAAASPYV

SEQ ID NO: 57 - protein, 15 aa, Artificial Sequence
  Id91 epitope 39
AAAASPYVAWMSVTA

SEQ ID NO: 58 - protein, 15 aa, Artificial Sequence
  Id91 epitope 40
VAWMSVTAGQAQLTA

SEQ ID NO: 59 - protein, 15 aa, Artificial Sequence
  Id91 epitope 41
AGQAQLTAAQVRVAA

SEQ ID NO: 60 - protein, 15 aa, Artificial Sequence
  Id91 epitope 42
AAQVRVAAAAYETAY

SEQ ID NO: 61 - protein, 15 aa, Artificial Sequence
  Id91 epitope 43
AAAYETAYRLTVPPP

SEQ ID NO: 62 - protein, 15 aa, Artificial Sequence
  Id91 epitope 44
YRLTVPPPVIAENRT

SEQ ID NO: 63 - protein, 15 aa, Artificial Sequence
  Id91 epitope 45
PVIAENRTELMTLTA

SEQ ID NO: 64 - protein, 15 aa, Artificial Sequence
  Id91 epitope 46
TELMTLTATNLLGQN

SEQ ID NO: 65 - protein, 15 aa, Artificial Sequence
  Id91 epitope 47
ATNLLGQNTPAIEAN

SEQ ID NO: 66 - protein, 15 aa, Artificial Sequence
  Id91 epitope 48
NTPAIEANQAAYSQM

SEQ ID NO: 67 - protein, 15 aa, Artificial Sequence
  Id91 epitope 49
NQAAYSQMWGQDAEA

SEQ ID NO: 68 - protein, 15 aa, Artificial Sequence
  Id91 epitope 50
MWGQDAEAMYGYAAT

SEQ ID NO: 69 - protein, 15 aa, Artificial Sequence
  Id91 epitope 51
AMYGYAATAATATEA

SEQ ID NO: 70 - protein, 15 aa, Artificial Sequence
  Id91 epitope 52
TAATATEALLPFEDA

SEQ ID NO: 71 - protein, 15 aa, Artificial Sequence
  Id91 epitope 53
ALLPFEDAPLITNPG

SEQ ID NO: 72 - protein, 15 aa, Artificial Sequence
  Id91 epitope 54
APLITNPGGLLEQAV

SEQ ID NO: 73 - protein, 15 aa, Artificial Sequence
  Id91 epitope 55
GGLLEQAVAVEEAID

SEQ ID NO: 74 - protein, 15 aa, Artificial Sequence
  Id91 epitope 56
VAVEEAIDTAAANQL

SEQ ID NO: 75 - protein, 15 aa, Artificial Sequence
  Id91 epitope 57
DTAAANQLMNNVPQA

SEQ ID NO: 76 - protein, 15 aa, Artificial Sequence
  Id91 epitope 58
LMNNVPQALQQLAQP

SEQ ID NO: 77 - protein, 15 aa, Artificial Sequence
  Id91 epitope 59
ALQQLAQPAQGVVPS

SEQ ID NO: 78 - protein, 15 aa, Artificial Sequence
  Id91 epitope 60
PAQGVVPSSKLGGLW

SEQ ID NO: 79 - protein, 15 aa, Artificial Sequence
  Id91 epitope 61
SSKLGGLWTAVSPHL

SEQ ID NO: 80 - protein, 15 aa, Artificial Sequence
  Id91 epitope 62
WTAVSPHLSPLSNVS

SEQ ID NO: 81 - protein, 15 aa, Artificial Sequence
  Id91 epitope 63
LSPLSNVSSIANNHM

SEQ ID NO: 82 - protein, 15 aa, Artificial Sequence
  Id91 epitope 64
SSIANNHMSMMGTGV

SEQ ID NO: 83 - protein, 15 aa, Artificial Sequence
  Id91 epitope 65
MSMMGTGVSMTNTLH

SEQ ID NO: 84 - protein, 15 aa, Artificial Sequence
  Id91 epitope 66
VSMTNTLHSMLKGLA

SEQ ID NO: 85 - protein, 16 aa, Artificial Sequence
  Id91 epitope 67
HSMLKGLAPAAAQAVE

SEQ ID NO: 86 - protein, 15 aa, Artificial Sequence
  Id91 epitope 68
PAAAQAVETAAENGV

SEQ ID NO: 87 - protein, 15 aa, Artificial Sequence
  Id91 epitope 69
ETAAENGVWAMSSLG

SEQ ID NO: 88 - protein, 15 aa, Artificial Sequence
  Id91 epitope 70
VWAMSSLGSQLGSSL

SEQ ID NO: 89 - protein, 15 aa, Artificial Sequence
  Id91 epitope 71
GSQLGSSLGSSGLGA

SEQ ID NO: 90 - protein, 15 aa, Artificial Sequence
  Id91 epitope 72
LGSSGLGAGVAANLG

SEQ ID NO: 91 - protein, 15 aa, Artificial Sequence
  Id91 epitope 73
AGVAANLGRAASVGS

SEQ ID NO: 92 - protein, 15 aa, Artificial Sequence
  Id91 epitope 74
GRAASVGSLSVPPAW

SEQ ID NO: 93 - protein, 15 aa, Artificial Sequence
  Id91 epitope 75
SLSVPPAWAAANQAV

SEQ ID NO: 94 - protein, 15 aa, Artificial Sequence
  Id91 epitope 76
WAAANQAVTPAARAL

SEQ ID NO: 95 - protein, 15 aa, Artificial Sequence
  Id91 epitope 77
VTPAARALPLTSLTS

SEQ ID NO: 96 - protein, 15 aa, Artificial Sequence
  Id91 epitope 78
LPLTSLTSAAQTAPG

SEQ ID NO: 97 - protein, 15 aa, Artificial Sequence
  Id91 epitope 79
SAAQTAPGHMLGGLP

SEQ ID NO: 98 - protein, 15 aa, Artificial Sequence
  Id91 epitope 80
GHMLGGLPLGHSVNA

SEQ ID NO: 99 - protein, 15 aa, Artificial Sequence
  Id91 epitope 81
PLGHSVNAGSGINNA

SEQ ID NO: 100 - protein, 15 aa, Artificial Sequence
  Id91 epitope 82
AGSGINNALRVPARA

SEQ ID NO: 101 - protein, 15 aa, Artificial Sequence
  Id91 epitope 83
ALRVPARAYAIPRTP

SEQ ID NO: 102 - protein, 15 aa, Artificial Sequence
  Id91 epitope 84
AYAIPRTPAAGFSRP

SEQ ID NO: 103 - protein, 15 aa, Artificial Sequence
  Id91 epitope 85
PAAGFSRPGLPVEYL

SEQ ID NO: 104 - protein, 15 aa, Artificial Sequence
  Id91 epitope 86
PGLPVEYLQVPSPSM

SEQ ID NO: 105 - protein, 15 aa, Artificial Sequence
  Id91 epitope 87
LQVPSPSMGRDIKVQ

SEQ ID NO: 106 - protein, 15 aa, Artificial Sequence
  Id91 epitope 88
MGRDIKVQFQSGGNN

SEQ ID NO: 107 - protein, 15 aa, Artificial Sequence
  Id91 epitope 89
QFQSGGNNSPAVYLL

SEQ ID NO: 108 - protein, 15 aa, Artificial Sequence
  Id91 epitope 90
NSPAVYLLDGLRAQD

SEQ ID NO: 109 - protein, 15 aa, Artificial Sequence
  Id91 epitope 91
LDGLRAQDDYNGWDI

SEQ ID NO: 110 - protein, 15 aa, Artificial Sequence
  Id91 epitope 92
DDYNGWDINTPAFEW

SEQ ID NO: 111 - protein, 15 aa, Artificial Sequence
  Id91 epitope 93
INTPAFEWYYQSGLS

SEQ ID NO: 112 - protein, 15 aa, Artificial Sequence
  Id91 epitope 94
WYYQSGLSIVMPVGG

SEQ ID NO: 113 - protein, 15 aa, Artificial Sequence
  Id91 epitope 95
SIVMPVGGQSSFYSD

SEQ ID NO: 114 - protein, 15 aa, Artificial Sequence
  Id91 epitope 96
GQSSFYSDWYSPACG

SEQ ID NO: 115 - protein, 15 aa, Artificial Sequence
  Id91 epitope 97
DWYSPACGKAGCQTY

SEQ ID NO: 116 - protein, 15 aa, Artificial Sequence
  Id91 epitope 98
GKAGCQTYKWETFLT

SEQ ID NO: 117 - protein, 15 aa, Artificial Sequence
  Id91 epitope 99
YKWETFLTSELPQWL

SEQ ID NO: 118 - protein, 15 aa, Artificial Sequence
  Id91 epitope 100
TSELPQWLSANRAVK

SEQ ID NO: 119 - protein, 15 aa, Artificial Sequence
  Id91 epitope 101
LSANRAVKPTGSAAI

SEQ ID NO: 120 - protein, 15 aa, Artificial Sequence
  Id91 epitope 102
KPTGSAAIGLSMAGS

SEQ ID NO: 121 - protein, 15 aa, Artificial Sequence
  Id91 epitope 103
IGLSMAGSSAMILAA

SEQ ID NO: 122 - protein, 15 aa, Artificial Sequence
  Id91 epitope 104
SSAMILAAYHPQQFI

SEQ ID NO: 123 - protein, 15 aa, Artificial Sequence
  Id91 epitope 105
AYHPQQFIYAGSLSA

SEQ ID NO: 124 - protein, 15 aa, Artificial Sequence
  Id91 epitope 106
IYAGSLSALLDPSQG

SEQ ID NO: 125 - protein, 15 aa, Artificial Sequence
  Id91 epitope 107
ALLDPSQGMGPSLIG

SEQ ID NO: 126 - protein, 15 aa, Artificial Sequence
  Id91 epitope 108
GMGPSLIGLAMGDAG

SEQ ID NO: 127 - protein, 15 aa, Artificial Sequence
  Id91 epitope 109
GLAMGDAGGYKAADM

SEQ ID NO: 128 - protein, 15 aa, Artificial Sequence
  Id91 epitope 110
GGYKAADMWGPSSDP

SEQ ID NO: 129 - protein, 15 aa, Artificial Sequence
  Id91 epitope 111
MWGPSSDPAWERNDP

SEQ ID NO: 130 - protein, 15 aa, Artificial Sequence
  Id91 epitope 112
PAWERNDPTQQIPKL

SEQ ID NO: 131 - protein, 15 aa, Artificial Sequence
  Id91 epitope 113
PTQQIPKLVANNTRL

SEQ ID NO: 132 - protein, 15 aa, Artificial Sequence
  Id91 epitope 114
LVANNTRLWVYCGNG

SEQ ID NO: 133 - protein, 15 aa, Artificial Sequence
  Id91 epitope 115
LWVYCGNGTPNELGG

SEQ ID NO: 134 - protein, 15 aa, Artificial Sequence
  Id91 epitope 116
GTPNELGGANIPAEF

SEQ ID NO: 135 - protein, 15 aa, Artificial Sequence
  Id91 epitope 117
GANIPAEFLENFVRS

SEQ ID NO: 136 - protein, 15 aa, Artificial Sequence
  Id91 epitope 118
FLENFVRSSNLKFQD

SEQ ID NO: 137 - protein, 15 aa, Artificial Sequence
  Id91 epitope 119
SSNLKFQDAYNAAGG

SEQ ID NO: 138 - protein, 15 aa, Artificial Sequence
  Id91 epitope 120
DAYNAAGGHNAVFNF

SEQ ID NO: 139 - protein, 15 aa, Artificial Sequence
  Id91 epitope 121
GHNAVFNFPPNGTHS

SEQ ID NO: 140 - protein, 15 aa, Artificial Sequence
  Id91 epitope 122
FPPNGTHSWEYWGAQ

SEQ ID NO: 141 - protein, 15 aa, Artificial Sequence
  Id91 epitope 123
SWEYWGAQLNAMKGD

SEQ ID NO: 142 - protein, 15 aa, Artificial Sequence
  Id91 epitope 124
QLNAMKGDLQSSLGA

SEQ ID NO: 143 - protein, 15 aa, Artificial Sequence
  Id91 epitope 125
AMKGDLQSSLGAGKL